European Patent Specification EP 3 999 085 B1, published March 12, 2025. Title: METHODS AND PRODUCTS FOR TREATMENT OF GASTROINTESTINAL DISORDERS. Applicant: Crestovo Holdings LLC Millennium Pharmaceuticals, Inc. The sequence listing filed with the application follows.

SEQUENCE LISTING (37 sequences)

SEQ ID NO: 1 - DNA, 1509 bp, Artificial Sequence
  Synthetic Polynucleotide
tataaagagtttgatcctggctcaggacgaacgctggcggcgcgcctaacacatgcaagtcgaacgagcgagagagagcttgctttctcgagcgagtggcgaacgggtgagtaacgcgtgaggaacctgcctcaaagagggggacaacagttggaaacgactgctaataccgcataagcccacggctcggcatcgagcagagggaaaaggagcaatccgctttgagatggcctcgcgtccgattagctagttggtgaggtaacggcccaccaaggcaacgatcggtagccggactgagaggttgaacggccacattgggactgagacacggcccagactcctacgggaggcagcagtggggaatattgcacaatgggggaaaccctgatgcagcgacgccgcgtggaggaagaaggtcttcggattgtaaactcctgttgttggggaagataatgacggtacccaacaaggaagtgacggctaactacgtgccagcagccgcggtaaaacgtaggtcacaagcgttgtccggaattactgggtgtaaagggagcgcaggcgggaagacaagttggaagtgaaatctatgggctcaacccataaactgctttcaaaactgtttttcttgagtagtgcagaggtaggcggaattcccggtgtagcggtggaatgcgtagatatcgggaggaacaccagtggcgaaggcggcctactgggcaccaactgacgctgaggctcgaaagtgtgggtagcaaacaggattagataccctggtagtccacaccgtaaacgatgattactaggtgttggaggattgaccccttcagtgccgcagttaacacaataagtaatccacctggggagtacgaccgcaaggttgaaactcaaaggaattgacgggggcccgcacaagcagtggagtatgtggtttaattcgacgcaacgcgaagaaccttaccaagtcttgacatcccttgacagacatagaaatatgtaatctcttcggagcaaggagacaggtggtgcatggttgtcgtcagctcgtgtcgtgagatgttgggttaagtcccgcaacgagcgcaacccttatggtcagttactacgcaagaggactctggccagactgccgttgacaaaacggaggaaggtggggatgacgtcaaatcatcatgccctttatgacttgggctacacacgtactacaatggcgttaaacaaagagaagcaagaccgcgaggtggagcaaaactcagaaacaacgtcccagttcggactgcaggctgcaactcgcctgcacgaagtcggaattgctagtaatcgtggatcagcatgccacggtgaatacgttcccgggccttgtacacaccgcccgtcacaccatgagagccggggggacccgaagtcggtagtctaaccgcaaggaggacgccgccgaaggtaaaactggtgattggggtgaagtcgtaacaaggtagccgtaggagaacctgcggctggatcacctccttt

SEQ ID NO: 2 - DNA, 1381 bp, Artificial Sequence
  Synthetic Polynucleotide
ggggtatagcccatggaaacgtggattaacaccccatagtacttttatcctgcatgggatgtgagttaaatgttcaaggtatcggatgggcatgcgtcctattagttagttggcggggtaacagcccaccaagacgatgataggtaggggttctgagaggaaggtcccccacattggaactgagacacggtccaaactcctacgggaggcagcagtgaggaatattggtcaatggacgtaagtctgaaccagccaagtcgcgtgagggaagactgccctatgggttgtaaacctcttttataagggaagaataagttctacgtgtagaatgatgcctgtaccttatgaataagcatcggctaactccgtgccagcagccgcggtaatacggaggatgcgagcgttatccggatttattgggtttaaagggtgcgtaggcggtttattaagttagtggttaaatatttgagctaaactcaattgtgccattaatactggtaaactggagtacagacgaggtaggcggaataagttaagtagcggtgaaatgcatagatataacttagaactccgatagcgaaggcagcttaccagactgtaactgacgctgatgcacgagagcgtgggtagcgaacaggattagataccctggtagtccacgccgtaaacgatgctcactggttctgtgcgatatattgtacgggattaagcgaaagtattaagtgagccacctggggagtacgtcggcaacgatgaaactcaaaggaattgacgggggcccgcacaagcggaggaacatgtggtttaattcgatgatacgcgaggaaccttacctgggtttaaatgggaaatgccgtatttggaaacagatattctcttcggagcgtttttcaaggtgctgcatggttgtcgtcagctcgtgccgtgaggtgtcgggttaagtcccataacgagcgcaacccttaccgttagttgctagcatgtaatgatgagcactctaacgggactgccaccgtaaggtgagaggaaggcggggatgacgtcaaatcagcacggcccttacacccagggctacacacgtgttacaatggccggtacagagggccgctaccaggtgactggatgccaatctcaaaagccggtcgtagttcggattggagtctgtaacccgactccatgaagttggattcgctagtaatcgcgcatcagccatggcgcggtgaatacgttcccgggccttgtacacaccgcccgtcaagccatggaagccgggggtgcctgaagtccgtaaccgcgaggatcggcctagggcaaaactggtaactggggctaagtcgtaacaaggtagccgtaccggaaggtgcggctggaacacctcctt

SEQ ID NO: 3 - DNA, 1299 bp, Artificial Sequence
  Synthetic Polynucleotide
tggtacaggatggacccgcgtctgattagctggttggtgaggtaacggctcaccaaggcgacgatcagtagccggcttgagagagtgaacggccacattgggactgagacacggcccaaactcctacgggaggcagcagtggggaatattgcacaatgggggaaaccctgatgcagcgacgccgcgtgagtgaagaagtatctcggtatgtaaagctctatcagcagggaagaaaatgacggtacctgactaagaagccccggctaactacgtgccagcagccgcggtaatacgtagggggcaagcgttatccggaattactgggtgtaaagggtgcgtaggtggtatggcaagtcagaagtgaaaacccagggcttaactctgggactgcttttgaaactgtcagactagagtgcaggagaggtaagcggaattcctagtgtagcggtgaaatgcgtagatattaggaggaacatcagtggcgaaggcggcttactggactgaaactgacactgaggcacgaaagcgtggggagcaaacaggattagataccctggtagtccacgccgtaaacgatgaatactaggtgtcggggccgtagaggcttcggtgccgcagccaacgcagtaagtattccacctggggagtacgttcgcaagaatgaaactcaaaggaattgacggggacccgcacaagcggtggagcatgtggtttaattcgaagcaacgcgaagaaccttacctggtcttgacatccttctgaccggtccttaaccggacttttccttcgggacaggagtgacaggtggtgcatggttgtcgtcagctcgtgtcgtgagatgttgggttaagtcccgcaacgagcgcaacccctatctttagtagccagcatataaggtgggcactctagagagactgccagggataacctggaggaaggtggggacgacgtcaaatcatcatgccccttatgaccagggctacacacgtgctacaatggcgtaaacagagggaagcagcctcgtgagagtgagcaaatcccaaaaataacgtctcagttcggattgtagtctgcaactcgactacatgaagctggaatcgctagtaatcgcgaatcagaatgtcgcggtgaatacgttcccgggtcttgtacacaccgcccgtcacaccatgggagtcagtaacgcccgaagtcagtgacccaaccgtaaggagggagctgccgaaggcgggaccgataactggggtgaagtcgtaacaaggtagccgtatcggaaggtgcggctggatcacctccttt

SEQ ID NO: 4 - DNA, 800 bp, Artificial Sequence
  Synthetic Polynucleotide
tgtgtatcgccgacaacgagttatcatcgtttactgcgtggactaccagggtatctaatcctgtttgctccccacgctttcgtgcctcaacgtcagatatagtttggtaagctgccttcgcaatcggtgttctgtatgatctctaagcatttcaccgctacaccatacattccgcctaccgcaactactctctagtctaacagtattagaggcagttccggagttaagccccgggatttcacctctaacttatcaaaccgcctacgcaccctttaaacccaataaatccggataacgcttgaatcctccgtattaccgcggctgctggcacggagttagccgatccttattcgtacgatactttcagtcacctacacgtaggtgagtttaccctcgtacaaaagcagtttacaactcatagagccgtcttcctgcacgcggcatggctggttcagacttgcgtccattgaccaatattcctcactgctgcctcccgtaggagtctgatccgtgtctcagtaccagtgtggggggttaacctctcagtccccctatgtatcgttgccttggtgagccgttacctcaccaactagctaatacaacgcatgtccatctataaccaccggagttttcaacccggagagatgcctctccgaatattatggggaattagtaccaatttctcagtgttatgcccctgttataggtaggttacatacgcgttacgcacccgtgcgccggtcgccggcaattgaagcaagcttcaatcccgatgcccctcgacttgcatgtgttaggcc

SEQ ID NO: 5 - DNA, 1527 bp, Artificial Sequence
  Synthetic Polynucleotide
cgaagagtttgatcctggctcaggatgaacgctagcgacaggcttaacacatgcaagtcgaggggcagcatgatttgtagcaatacagattgatggcgaccggcgcacgggtgagtaacgcgtatgcaacttacctatcagagggggatagcccggcgaaagtcggattaataccccataaaacaggggtcccgcatgggaatatttgttaaagattcatcgctgatagataggcatgcgttccattaggcagttggcggggtaacggcccaccaaaccgacgatggataggggttctgagaggaaggtcccccacattggtactgagacacggaccaaactcctacgggaggcagcagtgaggaatattggtcaatggccgagaggctgaaccagccaagtcgcgtgaaggaagaaggatctatggtttgtaaacttcttttataggggaataaagtggaggacgtgtccttttttgtatgtaccctatgaataagcatcggctaactccgtgccagcagccgcggtaatacggaggatgcgagcgttatccggatttattgggtttaaagggtgcgtaggtggtgatttaagtcagcggtgaaagtttgtggctcaaccataaaattgccgttgaaactgggttacttgagtgtgtttgaggtaggcggaatgcgtggtgtagcggtgaaatgcatagatatcacgcagaactccgattgcgaaggcagcttactaaaccataactgacactgaagcacgaaagcgtggggatcaaacaggattagataccctggtagtccacgcagtaaacgatgattactaggagtttgcgatacaatgtaagctctacagcgaaagcgttaagtaatccacctggggagtacgccggcaacggtgaaactcaaaggaattgacgggggcccgcacaagcggaggaacatgtggtttaattcgatgatacgcgaggaaccttacccgggtttgaacgtagtctgaccggagtggaaacactctttctagcaatagcagattacgaggtgctgcatggttgtcgtcagctcgtgccgtgaggtgtcggcttaagtgccataacgagcgcaacccttatcactagttactaacaggtgaagctgaggactctggtgagactgccagcgtaagctgtgaggaaggtggggatgacgtcaaatcagcacggcccttacatccggggcgacacacgtgttacaatggcatggacaaagggcagctacctggcgacaggatgctaatctccaaaccatgtctcagttcggatcggagtctgcaactcgactccgtgaagctggattcgctagtaatcgcgcatcagccatggcgcggtgaatacgttcccgggccttgtacacaccgcccgtcaagccatgggagccgggggtacctgaagtccgtaaccgcaaggatcggcctagggtaaaactggtgactggggctaagtcgtaacaaggtagccgtaccggaaggtgcggctggaacacctccttt

SEQ ID NO: 6 - DNA, 1529 bp, Artificial Sequence
  Synthetic Polynucleotide
aacgagagtttgatcctggctcaggatgaacgctggcggcgtgcttaacacatgcaagtcgagcgaagcactttggaaagattcttcggatgatttcctttgtgactgagcggcggacgggtgagtaacgcgtgggtaacctgcctcatacagggggataacagttagaaatgactgctaataccgcataagaccacggtaccgcatggtacagtggtaaaaactccggtggtatgagatggacccgcgtctgattaggtagttggtggggtaacggcctaccaagccgacgatcagtagccgacctgagagggtgaccggccacattgggactgagacacggcccagactcctacgggaggcagcagtggggaatattgcacaatggaggaaactctgatgcagcgacgccgcgtgaaggatgaagtatttcggtatgtaaacttctatcagcagggaagaaaatgacggtacctgactaagaagccccggctaactacgtgccagcagccgcggtaatacgtagggggcaagcgttatccggatttactgggtgtaaagggagcgtagacggcacggcaagccagatgtgaaagcccggggctcaaccccgggactgcatttggaactgctgagctagagtgtcggagaggcaagtggaattcctagtgtagcggtgaaatgcgtagatattaggaggaacaccagtggcgaaggcggcttgctggacgatgactgacgttgaggctcgaaagcgtggggagcaaacaggattagataccctggtagtccacgccgtaaacgatgactgctaggtgtcgggtggcaaagccattcggtgccgcagctaacgcaataagcagtccacctggggagtacgttcgcaagaatgaaactcaaaggaattgacggggacccgcacaagcggtggagcatgtggtttaattcgaagcaacgcgaagaaccttacctgatcttgacatcccgatgaccgcttcgtaatggaagtttttcttcggaacatcggtgacaggtggtgcatggttgtcgtcagctcgtgtcgtgagatgttgggttaagtcccgcaacgagcgcaacccctatcttcagtagccagcaggttaagctgggcactctggagagactgccagggataacctggaggaaggtggggatgacgtcaaatcatcatgccccttatgaccagggctacacacgtgctacaatggcgtaaacaaagagaagcgaactcgcgagagtaagcaaatctcaaaaataacgtctcagttcggattgtagtctgcaactcgactacatgaagctggaatcgctagtaatcgcagatcagaatgctgcggtgaatacgttcccgggtcttgtacacaccgcccgtcacaccatgggagtcagtaacgcccgaagtcagtgacccaaccgtaaggagggagctgccgaaggtgggaccgataactggggtgaagtcgtaacaaggtagccgtatcggaaggtgcggctggatcacctccttt

SEQ ID NO: 7 - DNA, 1509 bp, Artificial Sequence
  Synthetic Polynucleotide
tataaagagtttgatcctggctcaggacgaacgctggcggcgcgcctaacacatgcaagtcgaacgagagagaaggagcttgcttcttcgatcgagtggcgaacgggtgagtaacgcgtgaggaacctgcctcaaagagggggacaacagttggaaacgactgctaataccgcataagcccacgggtcggcatcgaccagagggaaaaggagcaatccgctttgagatggcctcgcgtccgattagctagttggtgaggtaatggcccaccaaggcgacgatcggtagccggactgagaggttgaacggccacattgggactgagacacggcccagactcctacgggaggcagcagtggggaatattgcacaatgggggaaaccctgatgcagcgacgccgcgtggaggaagaaggtcttcggattgtaaactcctgttgttgaggaagataatgacggtactcaacaaggaagtgacggctaactacgtgccagcagccgcggtaaaacgtaggtcacaagcgttgtccggaattactgggtgtaaagggagcgcaggcgggaagacaagttggaagtgaaatccatgggctcaacccatgaactgctttcaaaactgtttttcttgagtagtgcagaggtaggcggaattcccggtgtagcggtggaatgcgtagatatcgggaggaacaccagtggcgaaggcggcctactgggcaccaactgacgctgaggctcgaaagtgtgggtagcaaacaggattagataccctggtagtccacaccgtaaacgatgattactaggtgttggaggattgaccccttcagtgccgcagttaacacaataagtaatccacctggggagtacgaccgcaaggttgaaactcaaaggaattgacgggggcccgcacaagcagtggagtatgtggtttaattcgacgcaacgcgaagaaccttaccaagtcttgacatcctgcgacggacatagaaatatgtctttccttcgggacgcagagacaggtggtgcatggttgtcgtcagctcgtgtcgtgagatgttgggttaagtcccgcaacgagcgcaacccttatggtcagttactacgcaagaggactctggccagactgccgttgacaaaacggaggaaggtggggatgacgtcaaatcatcatgccctttatgacttgggctacacacgtactacaatggcgttaaacaaagagaagcaagaccgcgaggtggagcaaaactcagaaacaacgtcccagttcggactgcaggctgcaactcgcctgcacgaagtcggaattgctagtaatcgtggatcagcatgccacggtgaatacgttcccgggccttgtacacaccgcccgtcacaccatgagagccggggggacccgaagtcggtagtctaaccgcaaggaggacgccgccgaaggtaaaactggtgattggggtgaagtcgtaacaaggtagccgtaggagaacctgcggctggatcacctccttt

SEQ ID NO: 8 - DNA, 1529 bp, Artificial Sequence
  Synthetic Polynucleotide
atgagagtttgatcctggctcaggatgaacgctggcggcgtgcttaacacatgcaagtcgaacgaagcactttatttgatttccttcgggactgattattttgtgactgagtggcggacgggtgagtaacgcgtgggtaacctgccttgtacagggggataacagttggaaacggctgctaataccgcataagcgcacagcatcgcatgatgcagtgtgaaaaactccggtggtataagatggacccgcgttggattagctagttggtgaggtaacggcccaccaaggcgacgatccatagccgacctgagagggtgaccggccacattgggactgagacacggcccaaactcctacgggaggcagcagtggggaatattgcacaatgggcgaaagcctgatgcagcgacgccgcgtgagcgaagaagtatttcggtatgtaaagctctatcagcagggaagataatgacggtacctgactaagaagcaccggctaaatacgtgccagcagccgcggtaatacgtatggtgcaagcgttatccggatttactgggtgtaaagggagcgcaggcggtgcggcaagtctgatgtgaaagcccggggctcaaccccggtactgcattggaaactgtcgtactagagtgtcggaggggtaagcggaattcctagtgtagcggtgaaatgcgtagatattaggaggaacaccagtggcgaaggcggcttactggacgataactgacgctgaggctcgaaagcgtggggagcaaacaggattagataccctggtagtccacgccgtaaacgatgaatactaggtgttgggaagcattgcttctcggtgccgtcgcaaacgcagtaagtattccacctggggagtacgttcgcaagaatgaaactcaaaggaattgacggggacccgcacaagcggtggagcatgtggtttaattcgaagcaacgcgaagaaccttaccaagtcttgacatccttctgaccggtacttaaccgtaccttctcttcggagcaggagtgacaggtggtgcatggttgtcgtcagctcgtgtcgtgagatgttgggttaagtcccgcaacgagcgcaacccttatctttagtagccagcggtttggccgggcactctagagagactgccagggataacctggaggaaggcggggatgacgtcaaatcatcatgccccttatgacttgggctacacacgtgctacaatggcgtaaacaaagggaagcaaagctgtgaagccgagcaaatctcaaaaataacgtctcagttcggactgtagtctgcaacccgactacacgaagctggaatcgctagtaatcgcagatcagaatgctgcggtgaatacgttcccgggtcttgtacacaccgcccgtcacaccatgggagttgggaatgcccgaagccagtgacctaaccgaaaggaaggagctgtcgaaggcaggctcgataactggggtgaagtcgtaacaaggtagccgtatcggaaggtgcggctggatcacctccttt

SEQ ID NO: 9 - DNA, 1118 bp, Artificial Sequence
  Synthetic Polynucleotide
aacggccacattgggactgagacacggcccagactcctacgggaggcagcagtggggaatattgcacaatgggggaaaccctgatgcagcgacgccgcgtgaaggaagaagtatctcggtatgtaaacttctatcagcagggaagatagtgacggtacctgactaagaagccccggctaactacgtgccagcagccgcggtaatacgtagggggcaagcgttatccggatttactgggtgtaaagggagcgtagacggactggcaagtctgatgtgaaaggcgggggctcaacccctggactgcattggaaactgttagtcttgagtgccggagaggtaagcggaattcctagtgtagcggtgaaatgcgtagatattaggaggaacaccagtggcgaaggcggcttactggacggtaactgacgttgaggctcgaaagcgtggggagcaaacaggattagataccctggtagtccacgccgtaaacgatgaatactaggtgttggggagcaaagctcttcggtgccgccgcaaacgcattaagtattccacctggggagtacgttcgcaagaatgaaactcaaaggaattgacggggacccgcacaagcggtggagcatgtggtttaattcgaagcaacgcgaagaaccttaccaagtcttgacatccctctgaccgttccttaaccggaactttccttcgggacaggggagacaggtggtgcatggttgtcgtcagctcgtgtcgtgagatgttgggttaagtcccgcaacgagcgcaacccctatccccagtagccagcagtccggctgggcactctgaggagactgccagggataacctggaggaaggcggggatgacgtcaaatcatcatgccccttatgatttgggctacacacgtgctacaatggcgtaaacaaagggaagcaagcctgcgaaggtaagcaaatcccaaaaataacgtcccagttcggactgcagtctgcaactcgactgcacgaagctggaatcgctagtaatcgcggatcagaatgccgcggtgaatacgttcccgggtcttgtacacaccgcccgtcacaccatgggagtcagtaacgcccgaagtcagtgacctaac

SEQ ID NO: 10 - DNA, 1531 bp, Artificial Sequence
  Synthetic Polynucleotide
aaaggaggtgatccagccgcaccttccgatacggctaccttgttacgacttcaccccagttacctgccccgccttcggcagctccctcctgttaaggttgggtcactgacttcgggcgttgctgactcccatggtgtgacgggcggtgtgtacaagacccgggaacgtattcaccgcggcattctgatccgcgattactagcgattccagcttcgtgtagtcgggttgcagactacagtccgaactgggacgttatttttgggatttgcttgccttcgcagggtcgcctccctttgtttacgccattgtagcacgtgtgtagcccaaatcataaggggcatgatgatttgacgtcatccccaccttcctccaggttatccctggcagtctccctagagtgcccaccacgacgtgctggctactaaggataagggttgcgctcgttgcgggacttaacccaacatctcacgacacgagctgacgacaaccatgcaccacctgtctctcttgccccgaagggaaggcgccgttacacgccggtcaagaggatgtcaagacttggtaaggttcttcgcgttgcttcgaattaaaccacatgctccaccgcttgtgcgggtccccgtcaattcctttgagtttcattcttgcgaacgtactccccaggtggaatgcttattgcgttagcggcggcaccgaagggctttgccccccgacacctagcattcatcgtttacggcgtggactaccagggtatctaatcctgtttgctccccacgctttcgagcctcaacgtcagttacagtccagtaagccgccttcgccactggtgttcctcctaatatctacgcatttcaccgctacactaggaattccacttacctctcctgcactccagcagcacagtttccaaagcagtcccggggttgggccccgggctttcactccagacttgcgtcgccgtctacgctccctttacacccagtaaatccggataacgcttgccccctacgtattaccgcggctgctggcacgtagttagccggggcttcttagtcaggtaccgtcattttcttccctgctgatagagctttacataccgagatacttcttcactcacgcggcgtcgctgcatcaggcttgcgcccattgtgcaatattccccactgctgcctcccgtaggagtttgggccgtgtctcagtcccaatgtggccggtcaccctctcaggtcggctactgatcgtcgctttggtgggccgttaccccgccaactggctaatcagacgcggatccatctcacaccacctgggtttttcacaccgtaccatgcggtactgtgcgcttatgcggtattagcagccatttctaactgttatcccccagtgtgaggcaggttatccacgcgttactcacccgtccgccactcagtcaaccaggaatccatccgaaaacttcatcctaatcgcttcgttcgacttgcatgtgttaggcacgccgccagcgttcatcctgagccaggatcaaactctcaaa

SEQ ID NO: 11 - DNA, 1523 bp, Artificial Sequence
  Synthetic Polynucleotide
atgaagagtttgatcctggctcaggatgaacgctagctacaggcttaacacatgcaagtcgaggggcagcatgaacttagcttgctaagtttgatggcgaccggcgcacgggtgagtaacacgtatccaacctgccgatgactcggggatagcctttcgaaagaaagattaatacccgatggcatagttcttccgcatggtggaactattaaagaatttcggtcatcgatggggatgcgttccattaggttgttggcggggtaacggcccaccaagccttcgatggataggggttctgagaggaaggtcccccacattggaactgagacacggtccaaactcctacgggaggcagcagtgaggaatattggtcaatggacgagagtctgaaccagccaagtagcgtgaaggatgactgccctatgggttgtaaacttcttttatacgggaataaagtgaggcacgtgtgcctttttgtatgtaccgtatgaataaggatcggctaactccgtgccagcagccgcggtaatacggaggatccgagcgttatccggatttattgggtttaaagggagcgtaggcggacgcttaagtcagttgtgaaagtttgcggctcaaccgtaaaattgcagttgatactgggtgtcttgagtacagtagaggcaggcggaattcgtggtgtagcggtgaaatgcttagatatcacgaagaactccgattgcgaaggcagcttgctggactgtaactgacgctgatgctcgaaagtgtgggtatcaaacaggattagataccctggtagtccacacagtaaacgatgaatactcgctgtttgcgatatacagtaagcggccaagcgaaagcgttaagtattccacctggggagtacgccggcaacggtgaaactcaaaggaattgacgggggcccgcacaagcggaggaacatgtggtttaattcgatgatacgcgaggaaccttacccgggcttgaattgcaactgaatgatgtggagacatgtcagccgcaaggcagttgtgaaggtgctgcatggttgtcgtcagctcgtgccgtgaggtgtcggcttaagtgccataacgagcgcaacccttatcgatagttaccatcaggttatgctggggactctgtcgagactgccgtcgtaagatgtgaggaaggtggggatgacgtcaaatcagcacggcccttacgtccggggctacacacgtgttacaatggggggtacagaaggcagctacacggcgacgtgatgctaatcccgaaagcctctctcagttcggattggagtctgcaacccgactccatgaagctggattcgctagtaatcgcgcatcagccacggcgcggtgaatacgttcccgggccttgtacacaccgcccgtcaagccatgaaagccgggggtacctgaagtgcgtaaccgcaaggagcgccctagggtaaaactggtgattggggctaagtcgtaacaaggtagccgtaccggaaggtgcggctggaacacctcctt

SEQ ID NO: 12 - DNA, 1319 bp, Artificial Sequence
  Synthetic Polynucleotide
tgattaaaggtattccggtagacgatggggatgcgttccattagatagtaggcggggtaacggcccacctagtcttcgatggataggggttctgagaggaaggtcccccacattggaactgagacacggtccaaactcctacgggaggcagcagtgaggaatattggtcaatgggcgcaggcctgaaccagccaagtagcgtgaaggatgactgccctatgggttgtaaacttcttttataaaggaataaagtcgggtatgtatacccgtttgcatgtactttatgaataaggatcggctaactccgtgccagcagccgcggtaatacggaggatccgagcgttatccggatttattgggtttaaagggagcgtagatggatgtttaagtcagttgtgaaagtttgcggctcaaccgtaaaattgcagttgatactggatatcttgagtgcagttgaggcaggcggaattcgtggtgtagcggtgaaatgcttagatatcacgaagaactccgattgcgaaggcagcctgctaagctgcaactgacattgaggctcgaaagtgtgggtatcaaacaggattagataccctggtagtccacacggtaaacgatgaatactcgctgtttgcgatatacggcaagcggccaagcgaaagcgttaagtattccacctggggagtacgccggcaacggtgaaactcaaaggaattgacgggggcccgcacaagcggaggaacatgtggtttaattcgatgatacgcgaggaaccttacccgggcttaaattgcagatgaattacggtgaaagccgtaagccgcaaggcatctgtgaaggtgctgcatggttgtcgtcagctcgtgccgtgaggtgtcggcttaagtgccataacgagcgcaacccttgttgtcagttactaacaggtttcgctgaggactctgacaagactgccatcgtaagatgtgaggaaggtggggatgacgtcaaatcagcacggcccttacgtccggggctacacacgtgttacaatggggggtacagagggccgctaccacgcgagtggatgccaatccccaaaacctctctcagttcggactggagtctgcaacccgactccacgaagctggattcgctagtaatcgcgcatcagccacggcgcggtgaatacgttcccgggccttgtacacaccgcccgtcaagccatgggagccgggggtacctgaagtgcgtaaccgcgaggagcgccctagggtaaaactggtgactggggctaagtcgtaacaaggtagccgtaccggaaggtgcggctggaacacctcctt

SEQ ID NO: 13 - DNA, 1523 bp, Artificial Sequence
  Synthetic Polynucleotide
atgaagagtttgatcctggctcaggatgaacgctagctacaggcttaacacatgcaagtcgaggggcagcatcatcaaagcttgctttgatggatggcgaccggcgcacgggtgagtaacacgtatccaacctgccgacaacactgggatagcctttcgaaagaaagattaataccggatggcatagttttcccgcatgggataattattaaagaatttcggttgtcgatggggatgcgttccattaggcagttggcggggtaacggcccaccaaaccaacgatggataggggttctgagaggaaggtcccccacattggaactgagacacggtccaaactcctacgggaggcagcagtgaggaatattggtcaatggacgagagtctgaaccagccaagtagcgtgaaggatgactgccctatgggttgtaaacttcttttatacgggaataaagtgagccacgtgtggctttttgtatgtaccgtatgaataaggatcggctaactccgtgccagcagccgcggtaatacggaggatccgagcgttatccggatttattgggtttaaagggagcgtaggcgggttgttaagtcagttgtgaaagtttgcggctcaaccgtaaaattgcagttgatactggcgaccttgagtgcaacagaggtaggcggaattcgtggtgtagcggtgaaatgcttagatatcacgaagaactccgattgcgaaggcagcttactggattgtaactgacgctgatgctcgaaagtgtgggtatcaaacaggattagataccctggtagtccacacagtaaacgatgaatactcgctgttggcgatatacggtcagcggccaagcgaaagcattaagtattccacctggggagtacgccggcaacggtgaaactcaaaggaattgacgggggcccgcacaagcggaggaacatgtggtttaattcgatgatacgcgaggaaccttacccgggcttaaattgcaactgacggaaccggaaacggttctttcttcggacagttgtgaaggtgctgcatggttgtcgtcagctcgtgccgtgaggtgtcggcttaagtgccataacgagcgcaacccttacgggtagttaccatcaggttatgctggggactctacccggactgccgtcgtaagatgtgaggaaggtggggatgacgtcaaatcagcacggcccttacgtccggggctacacacgtgttacaatggggggtacagaaggcagctacacggcgacgtggtgctaatcccaaaagcctctctcagttcggattggagtctgcaacccgactccatgaagctggattcgctagtaatcgcgcatcagccacggcgcggtgaatacgttcccgggccttgtacacaccgcccgtcaagccatgaaagccgggggtacctgaagtacgtaaccgcgaggagcgtcctagggtaaaactggtgattggggctaagtcgtaacaaggtagccgtaccggaaggtgcggctggaacacctcctt

SEQ ID NO: 14 - DNA, 1519 bp, Artificial Sequence
  Synthetic Polynucleotide
atgaagagtttgatcctggctcaggatgaacgctagctacaggcttaacacatgcaagtcgaggggcagcatgacctagcaataggttgatggcgaccggcgcacgggtgagtaacacgtatccaacctaccggttattccgggatagcctttcgaaagaaagattaataccggatagtataacgagaaggcatctttttgttattaaagaatttcgataaccgatggggatgcgttccattagtttgttggcggggtaacggcccaccaagacatcgatggataggggttctgagaggaaggtcccccacattggaactgagacacggtccaaactcctacgggaggcagcagtgaggaatattggtcaatggacgagagtctgaaccagccaagtagcgtgaaggatgactgccctatgggttgtaaacttcttttatatgggaataaagtgagccacgtgtggctttttgtatgtaccatacgaataaggatcggctaactccgtgccagcagccgcggtaatacggaggatccgagcgttatccggatttattgggtttaaagggagcgtaggcggactattaagtcagctgtgaaagtttgcggctcaaccgtaaaattgcagttgatactggtcgtcttgagtgcagtagaggtaggcggaattcgtggtgtagcggtgaaatgcttagatatcacgaagaactccgattgcgaaggcagcttactggactgtaactgacgctgatgctcgaaagtgtgggtatcaaacaggattagataccctggtagtccacacagtaaacgatgaatactcgctgtttgcgatatacagcaagcggccaagcgaaagcattaagtattccacctggggagtacgccggcaacggtgaaactcaaaggaattgacgggggcccgcacaagcggaggaacatgtggtttaattcgatgatacgcgaggaaccttacccgggcttaaattgcatctgaataatttggaaacagattagccgcaaggcagatgtgaaggtgctgcatggttgtcgtcagctcgtgccgtgaggtgtcggcttaagtgccataacgagcgcaacccttatctttagttactaacaggtcatgctgaggactctagagagactgccgtcgtaagatgtgaggaaggtggggatgacgtcaaatcagcacggcccttacgtccggggctacacacgtgttacaatggggggtacagaaggcagctacacagcgatgtgatgctaatcccaaaagcctctctcagttcggattggagtctgcaacccgactccatgaagctggattcgctagtaatcgcgcatcagccacggcgcggtgaatacgttcccgggccttgtacacaccgcccgtcaagccatgaaagccgggggtacctgaagtccgtaaccgtaaggagcggcctagggtaaaactggtaattggggctaagtcgtaacaaggtagccgtaccggaaggtgcggctggaacacctcctt

SEQ ID NO: 15 - DNA, 1521 bp, Artificial Sequence
  Synthetic Polynucleotide
atggagagtttgatcctggctcaggatgaacgctagcggcaggcctaacacatgcaagtcgaggggcatcacgaggtagcaatactttggtggcgaccggcgcacgggtgcgtaacgcgtatgtaacctacctataacaggggcataacactgagaaattggtactaattccccataatattcggagaggcatctctccgggttgaaaactccggtggttatagatggacatgcgttgtattagctagttggtgaggtaacggctcaccaaggcaacgatacatagggggactgagaggttaaccccccacactggtactgagacacggaccagactcctacgggaggcagcagtgaggaatattggtcaatggacgcaagtctgaaccagccatgccgcgtgcaggaagacggctctatgagttgtaaactgcttttgtacgagggtaaactcacctacgtgtaggtgactgaaagtatcgtacgaataaggatcggctaactccgtgccagcagccgcggtaatacggaggattcaagcgttatccggatttattgggtttaaagggtgcgtaggcggtttgataagttagaggtgaaatcccggggcttaactccggaactgcctctaatactgttagactagagagtagttgcggtaggcggaatgtatggtgtagcggtgaaatgcttagagatcatacagaacaccgattgcgaaggcagcttaccaaactatatctgacgttgaggcacgaaagcgtggggagcaaacaggattagataccctggtagtccacgcagtaaacgatgataactcgttgtcggcgatacacagtcggtgactaagcgaaagcgataagttatccacctggggagtacgttcgcaagaatgaaactcaaaggaattgacgggggcccgcacaagcggaggaacatgtggtttaattcgatgatacgcgaggaaccttacccgggcttgaaagttactgacgattctggaaacaggatttccctttggggcaggaaactaggtgctgcatggttgtcgtcagctcgtgccgtgaggtgtcgggttaagtcccataacgagcgcaacccctaccgttagttgccatcaggtcaagctgggcactctggcgggactgccggtgtaagccgagaggaaggtggggatgacgtcaaatcagcacggcccttacgtccggggctacacacgtgttacaatggtaggtacagagggtcgctactccgtgaggagatgccaatctcgaaagcctatctcagttcggattggaggctgaaacccgcctccatgaagttggattcgctagtaatcgcgcatcagccatggcgcggtgaatacgttcccgggccttgtacacaccgcccgtcaagccatggaagctgggggtgcctgaagttcgtgaccgcaaggagcgacctagggcaaaaccggtaactggggctaagtcgtaacaaggtagccgtaccggaaggtgcggctggaacacctccttt

SEQ ID NO: 16 - DNA, 1523 bp, Artificial Sequence
  Synthetic Polynucleotide
atgaagagtttgatcctggctcaggatgaacgctagctacaggcttaacacatgcaagtcgaggggcagcatgaacttagcttgctaagtttgatggcgaccggcgcacgggtgagtaacacgtatccaacctgccgatgactcggggatagcctttcgaaagaaagattaatacccgatggcatagttcttccgcatggtagaactattaaagaatttcggtcatcgatggggatgcgttccattaggttgttggcggggtaacggcccaccaagccttcgatggataggggttctgagaggaaggtcccccacattggaactgagacacggtccaaactcctacgggaggcagcagtgaggaatattggtcaatggacgagagtctgaaccagccaagtagcgtgaaggatgactgccctatgggttgtaaacttcttttatacgggaataaagtgaggcacgtgtgcctttttgtatgtaccgtatgaataaggatcggctaactccgtgccagcagccgcggtaatacggaggatccgagcgttatccggatttattgggtttaaagggagcgtaggcggacgcttaagtcagttgtgaaagtttgcggctcaaccgtaaaattgcagttgatactgggtgtcttgagtacagtagaggcaggcggaattcgtggtgtagcggtgaaatgcttagatatcacgaagaactccgattgcgaaggcagcttgctggactgtaactgacgctgatgctcgaaagtgtgggtatcaaacaggattagataccctggtagtccacacagtaaacgatgaatactcgctgtttgcgatatacagtaagcggccaagcgaaagcgttaagtattccacctggggagtacgccggcaacggtgaaactcaaaggaattgacgggggcccgcacaagcggaggaacatgtggtttaattcgatgatacgcgaggaaccttacccgggcttgaattgcaactgaatgatgtggagacatgtcagccgcaaggcagttgtgaaggtgctgcatggttgtcgtcagctcgtgccgtgaggtgtcggcttaagtgccataacgagcgcaacccttatcgatagttaccatcaggttatgctggggactctgtcgagactgccgtcgtaagatgtgaggaaggtggggatgacgtcaaatcagcacggcccttacgtccggggctacacacgtgttacaatggggggtacagaaggcagctacacggcgacgtgatgctaatccctaaagcctctctcagttcggattggagtctgcaacccgactccatgaagctggattcgctagtaatcgcgcatcagccacggcgcggtgaatacgttcccgggccttgtacacaccgcccgtcaagccatgaaagccgggggtacctgaagtgcgtaaccgcaaggagcgccctagggtaaaactggtgattggggctaagtcgtaacaaggtagccgtaccggaaggtgcggctggaacacctcctt

SEQ ID NO: 17 - DNA, 1527 bp, Artificial Sequence
  Synthetic Polynucleotide
acgagagtttgatcctggctcaggatgaacgctggcggcgtgcttaacacatgcaagtcgaacgaagcacctggatttgattcttcggatgaagatccttgtgactgagtggcggacgggtgagtaacgcgtgggtaacctgcctcatacagggggataacagttagaaatgactgctaataccgcataagaccacagggtcgcatgacctggtgggaaaaactccggtggtatgagatggacccgcgtctgattaggtagttggtggggtaacggcctaccaagccgacgatcagtagccgacctgagagggtgaccggccacattgggactgagacacggcccaaactcctacgggaggcagcagtggggaatattgcacaatgggggaaaccctgatgcagcgacgccgcgtgagcgaagaagtatttcggtatgtaaagctctatcagcagggaagaaaatgacggtacctgactaagaagcaccggctaaatacgtgccagcagccgcggtaatacgtatggtgcaagcgttatccggatttactgggtgtaaagggagcgtagacggctgtgtaagtctgaagtgaaagcccggggctcaaccccgggactgctttggaaactatgcagctagagtgtcggagaggtaagtggaattcccagtgtagcggtgaaatgcgtagatattgggaggaacaccagtggcgaaggcggcttactggacgatgactgacgttgaggctcgaaagcgtggggagcaaacaggattagataccctggtagtccacgccgtaaacgatgactactaggtgtcggggagcaaagctcttcggtgccgcagcaaacgcaataagtagtccacctggggagtacgttcgcaagaatgaaactcaaaggaattgacggggacccgcacaagcggtggagcatgtggtttaattcgaagcaacgcgaagaaccttacctgctcttgacatcccggtgaccggcatgtaatgatgccttttcttcggaacaccggtgacaggtggtgcatggttgtcgtcagctcgtgtcgtgagatgttgggttaagtcccgcaacgagcgcaacccttatcttcagtagccagcattttaggtgggcactctggagagactgccagggataacctggaggaaggtggggatgacgtcaaatcatcatgccccttatgagcagggctacacacgtgctacaatggcgtaaacaaagggaagcaaacctgtgagggtaagcaaatctcaaaaataacgtctcagttcggattgtagtctgcaactcgactacatgaagctggaatcgctagtaatcgcgaatcagcatgtcgcggtgaatacgttcccgggtcttgtacacaccgcccgtcacaccatgggagttggtaacgcccgaagtcagtgactcaaccgtaaggagagagctgccgaaggtgggaccgataactggggtgaagtcgtaacaaggtagccgtatcggaaggtgcggctggatcacctccttt

SEQ ID NO: 18 - DNA, 1521 bp, Artificial Sequence
  Synthetic Polynucleotide
atggagagtttgatcctggctcaggatgaacgctagcggcaggcctaacacatgcaagtcgaggggcagcacggtgtagcaatacactggtggcgaccggcgcacgggtgcgtaacgcgtatgcaacctacccataacagggggataacactgagaaattggtactaataccccataacatcaggaccggcatcggttctggttgaaaactccggtggttatggatgggcatgcgttgtattagctggttggtgaggtaacggctcaccaaggcaacgatacatagggggactgagaggttaaccccccacattggtactgagacacggaccaaactcctacgggaggcagcagtgaggaatattggtcaatggacgcaagtctgaaccagccatgccgcgtgcaggaagacggctctatgagttgtaaactgcttttgtacgagagtaaacgctcttacgtgtaagagcctgaaagtatcgtacgaataaggatcggctaactccgtgccagcagccgcggtaatacggaggatccaagcgttatccggatttattgggtttaaagggtgcgtaggcggtttgataagttagaggtgaaataccggtgcttaacaccggaactgcctctaatactgttgaactagagagtagttgcggtaggcggaatgtatggtgtagcggtgaaatgcttagagatcatacagaacaccgattgcgaaggcagcttaccaaactatatctgacgttgaggcacgaaagcgtggggagcaaacaggattagataccctggtagtccacgcagtaaacgatgataactcgctgtcggcgatacacggtcggcggctaagcgaaagcgataagttatccacctggggagtacgttcgcaagaatgaaactcaaaggaattgacgggggcccgcacaagcggaggaacatgtggtttaattcgatgatacgcgaggaaccttacccgggcttgaaagttactgacgattctggaaacaggatttcccttcggggcaggaaactaggtgctgcatggttgtcgtcagctcgtgccgtgaggtgtcgggttaagtcccataacgagcgcaacccctaccgttagttgccatcaggtcaagctgggcactctggcgggactgccggtgtaagccgagaggaaggtggggatgacgtcaaatcagcacggcccttacgtccggggctacacacgtgttacaatggtaggtacagagggcagctacccagtgatgggatgcgaatctcgaaagcctatctcagttcggatcggaggctgaaacccgcctccgtgaagttggattcgctagtaatcgcgcatcagccatggcgcggtgaatacgttcccgggccttgtacacaccgcccgtcaagccatggaagctgggggtgcctgaagttcgtgaccgcaaggagcgacctagggcaaaaccggtgactggggctaagtcgtaacaaggtagccgtaccggaaggtgcggctggaacacctccttt

SEQ ID NO: 19 - DNA, 1530 bp, Artificial Sequence
  Synthetic Polynucleotide
atgagagtttgatcctggctcaggatgaacgctggcggcgtgcttaacacatgcaagtcgaacgaagcactctatttgattttcttcggaaatgaagattttgtgactgagtggcggacgggtgagtaacgcgtgggtaacctgcctcatacagggggataacagttggaaacgactgctaataccgcataagcgcacaggatcacatgatccggtgtgaaaaactccggtggtatgagatggacccgcgtctgattagccagttggcagggtaacggcctaccaaagcgacgatcagtagccgacctgagagggtgaccggccacattgggactgagacacggcccaaactcctacgggaggcagcagtggggaatattgcacaatgggggaaaccctgatgcagcgacgccgcgtgagcgaagaagtatttcggtatgtaaagctctatcagcagggaagaagaatgacggtacctgactaagaagcaccggctaaatacgtgccagcagccgcggtaatacgtatggtgcaagcgttatccggatttactgggtgtaaagggagcgcaggcggtgcggcaagtctgatgtgaaagcccggggctcaaccccggtactgcattggaaactgtcgtactagagtgtcggaggggtaagtggaattcctagtgtagcggtgaaatgcgtagatattaggaggaacaccagtggcgaaggcggcttactggacgataactgacgctgaggctcgaaagcgtggggagcaaacaggattagataccctggtagtccacgccgtaaacgatgaatactaggtgtcggggagcattgctcttcggtgccgcagcaaacgcaataagtattccacctggggagtacgttcgcaagaatgaaactcaaaggaattgacggggacccgcacaagcggtggagcatgtggtttaattcgaagcaacgcgaagaaccttaccaagtcttgacatcccgatgacagggtatgtaatgtactttctcttcggagcatcggtgacaggtggtgcatggttgtcgtcagctcgtgtcgtgagatgttgggttaagtcccgcaacgagcgcaacccctgtccttagtagccagcggttcggccgggcactctagggagactgccagggataacctggaggaaggcggggatgacgtcaaatcatcatgccccttatgacttgggctacacacgtgctacaatggcgtaaacaaagggaagcggagccgtgaggccgagcaaatctcaaaaataacgtctcagttcggactgtagtctgcaacccgactacacgaagctggaatcgctagtaatcgcagatcagaatgctgcggtgaatacgttcccgggtcttgtacacaccgcccgtcacaccatgggagttggaaatgcccgaagtcagtgacccaaccgcaaggagggagctgccgaaggcaggttcgataactggggtgaagtcgtaacaaggtagccgtatcggaaggtgcggctggatcacctccttt

SEQ ID NO: 20 - DNA, 1509 bp, Artificial Sequence
  Synthetic Polynucleotide
atggagagtttgattctggctcagaacgaacgctggcggcgtggataagacatgcaagtcgaacgagagaattgctagcttgctaataattctctagtggcgcacgggtgagtaacacgtgagtaacctgcccccgagagcgggatagccctgggaaactgggattaataccgcatagtatcgaaagattaaagcagcaatgcgcttggggatgggctcgcggcctattagttagttggtgaggtaacggctcaccaaggcgatgacgggtagccggtctgagaggatgtccggccacactggaactgagacacggtccagacacctacgggtggcagcagtcgagaatcattcacaatgggggaaaccctgatggtgcgacgccgcgtgggggaatgaaggtcttcggattgtaaacccctgtcatgtgggagcaaattaaaaagatagtaccacaagaggaagagacggctaactctgtgccagcagccgcggtaatacagaggtctcaagcgttgttcggaatcactgggcgtaaagcgtgcgtaggctgtttcgtaagtcgtgtgtgaaaggcgcgggctcaacccgcggacggcacatgatactgcgagactagagtaatggagggggaaccggaattctcggtgtagcagtgaaatgcgtagatatcgagaggaacactcgtggcgaaggcgggttcctggacattaactgacgctgaggcacgaaggccaggggagcgaaagggattagatacccctgtagtcctggcagtaaacggtgcacgcttggtgtgcggggaatcgaccccctgcgtgccggagctaacgcgttaagcgtgccgcctggggagtacggtcgcaagattaaaactcaaagaaattgacggggacccgcacaagcggtggagtatgtggcttaattcgatgcaacgcgaagaaccttacctgggcttgacatgtaatgaacaacatgtgaaagcatgcgactcttcggaggcgttacacaggtgctgcatggccgtcgtcagctcgtgtcgtgagatgtttggttaagtccagcaacgagcgcaacccctgttgccagttaccagcacgtgaaggtggggactctggcgagactgcccagatcaactgggaggaaggtggggacgacgtcaggtcagtatggcccttatgcccagggctgcacacgtactacaatgcccagtacagagggggccgaagccgcgaggcggaggaaatcctaaaaactgggcccagttcggactgtaggctgcaacccgcctacacgaagccggaatcgctagtaatggcgcatcagctacggcgccgtgaatacgttcccgggtcttgtacacaccgcccgtcacatcatggaagccggtcgcacccgaagtatctgaagccaaccgcaaggaggcagggtcctaaggtgagactggtaactgggatgaagtcgtaacaaggtagccgtaggggaacctgcggctggatcacctccttt

SEQ ID NO: 21 - DNA, 1557 bp, Artificial Sequence
  Synthetic Polynucleotide
attggagagtttgatcctggctcaggacgaacgctggcggcgtgcctaacacatgcaagtcgaacggagaattttatttcggtagaattcttagtggcgaacgggtgagtaacgcgtaggcaacctgccctttagacggggacaacattccgaaaggagtgctaataccggatgtgatcatcgtgccgcatggcaggatgaagaaagatggcctctacaagtaagctatcgctaaaggatgggcctgcgtctgattagctagttggtagtgtaacggactaccaaggcgatgatcagtagccggtctgagaggatgaacggccacattgggactgagacacggcccaaactcctacgggaggcagcagtggggaatcttccgcaatggacgaaagtctgacggagcaacgccgcgtgagtgatgaaggatttcggtctgtaaagctctgttgtttatgacgaacgtgcagtgtgtgaacaatgcattgcaatgacggtagtaaacgaggaagccacggctaactacgtgccagcagccgcggtaatacgtaggtggcgagcgttgtccggaattattgggcgtaaagagcatgtaggcggcttaataagtcgagcgtgaaaatgcggggctcaaccccgtatggcgctggaaactgttaggcttgagtgcaggagaggaaaggggaattcccagtgtagcggtgaaatgcgtagatattgggaggaacaccagtggcgaaggcgcctttctggactgtgtctgacgctgagatgcgaaagccagggtagcgaacgggattagataccccggtagtcctggccgtaaacgatgggtactaggtgtaggaggtatcgaccccttctgtgccggagttaacgcaataagtaccccgcctggggagtacggccgcaaggttgaaactcaaaggaattgacgggggcccgcacaagcggtggagtatgtggtttaattcgacgcaacgcgaagaaccttaccaaggcttgacattgattgaacgctctagagatagagatttcccttcggggacaagaaaacaggtggtgcatggctgtcgtcagctcgtgtcgtgagatgttgggttaagtcccgcaacgagcgcaacccctatcctatgttaccagcaagtaaagttggggactcatgggagactgccagggacaacctggaggaaggcggggatgacgtcaagtcatcatgccccttatgtcttgggctacacacgtactacaatggtcggaaacagagggaagcgaagccgcgaggcagagcaaaccccagaaacccgatctcagttcggatcgcaggctgcaacccgcctgcgtgaagtcggaatcgctagtaatcgcaggtcagcatactgcggtgaatacgttcccgggccttgtacacaccgcccgtcacaccacgaaagttggtaacacccgaagccggtgaggtaacctataaggagccagccgtctaaggtggggccgatgattggggtgaagtcgtaacaaggtagccgtatcggaaggtgcggctggatcacctccttt

SEQ ID NO: 22 - DNA, 809 bp, Artificial Sequence
  Synthetic Polynucleotide
  misc_feature (631)..(631): n is a, c, g, or t
ctgagggggtcaatcccccaacacctagtaatcatcgtttacggcatggactaccagggtatctaatcctgtttgctacccatgctttcgagcctcagcgtcagttggtgcccagtagaccgccttcgccactggtgttcctcccgatatctacgcattccaccgctacaccgggaattccatctacctctgcactactcaagaaaaacagttttgaaagcaattcatgggttgagcccatggttttcacttccaacttgtcttcccgcctgcgctccctttacacccagtaattccggacaacgcttgcaccctacgttttaccgcggctgctggcacgtagttagccggtgctttcttgttaggtaccgtcattatcgtccctaacgacaggagtttacaatccgaaaaccttcttcctccacgcggcgtcgctgcatcagggtttcccccattgtgcaatatcccccactgctgcctcccgtaggagtctgggccgtgtctcagtcccaatgtggccgttcaacctctcagtccggctaccaatcgtcgccttggtgggccgttacctcaccaactagctaattggacgcgagtccatcctaaagcgaataaatccttttccctcagnaccatgcggtaccgtgggcttatgcggtattagcagtcgtttccaactgttgtcccccactctagggcaggttactcacgcgttactcacccgttcgccactaagcttaaaaagcaagctctctaagctccgttcgacttgcatgtgttaggcgcgccgccagcgttcgtcctgagcc

SEQ ID NO: 23 - DNA, 902 bp, Artificial Sequence
  Synthetic Polynucleotide
  misc_feature (796)..(796): n is a, c, g, or t
  misc_feature (825)..(825): n is a, c, g, or t
  misc_feature (838)..(838): n is a, c, g, or t
  misc_feature (841)..(841): n is a, c, g, or t
  misc_feature (881)..(881): n is a, c, g, or t
tgctttctcgagcgagtggcgaacgggtgagtaacgcgtgaggaacctgcctcaaagagggggacaacagttggaaacgactgctaataccgcataagcccacgacccggcatcgggtagagggaaaaggagcaatccgctttgagatggcctcgcgtccgattagctagttggtgaggtaacggcccaccaaggcgacgatcggtagccggactgagaggttgaacggccacattgggactgagacacggcccagactcctacgggaggcagcagtggggaatattgcacaatgggggaaaccctgatgcagcgacgccgcgtggaggaagaaggtcttcggattgtaaactcctgttgttgaggaagataatgacggtactcaacaaggaagtgacggctaactacgtgccagcagccgcggtaaaacgtaggtcacaagcgttgtccggaattactgggtgtaaagggagcgcaggcgggaaggcaagttggaagtgaaatccatgggctcaacccatgaactgctttcaaaactgtttttcttgagtagtgcagaggtaggcggaattcccggtgtagcggtggaatgcgtagatatcgggaggaacaccagtggcgaaggcggcctactgggcaccaactgacgctgaggctcgaaagtgtgggtagcaaacaggattagataccctggtagtccacactgtaaacgatgattactaggtgttggaggattgaccccttcagtgccgcagttaacacaataagtaatccacctggggagtacgaccgcaanggttgaaactcaaaggaattgacgggggnccgcacaagcagnggngtatgtggtttaattcgacgcaacgcgaagaaccttaccnagtcttgacatcctgcgacgg

SEQ ID NO: 24 - DNA, 1000 bp, Artificial Sequence
  Synthetic Polynucleotide
ataccttgatggcgaccggcgcacgggtgagtaacgcgtatgcaacctgcctgataccggggtatagcccatggaaacgtggattaacaccccatagtacttttatcctgcatgggatgtgagttaaatgttcaaggtatcggatgggcatgcgtcctattagttagttggcggggtaacagcccaccaagacgatgataggtaggggttctgagaggaaggtcccccacattggaactgagacacggtccaaacttctacgggaggcagcagtgaggaatattggtcaatggacgtaagtctgaaccagccaagtcgcgtgagggaagactgccctatgggttgtaaacctcttttataagggaagaataagttctacgtgtagaatgatgcctgtaccttatgaataagcatcggctaactccgtgccagcagccgcggtaatacggaggatgcgagcgttatccggatttattgggtttaaagggtgcgtaggcggtttattaagttagtggttaaatatttgagctaaactcaattgtgccattaatactggtaaactggagtacagacgaggtaggcggaataagttaagtagcggtgaaatgcatagatataacttagaactccgatagcgaaggcagcttaccagactgtaactgacgctgatgcacgagagcgtgggtagcgaacaggattagataccctggtagtccacgccgtaaacgatgctcactggttctgtgcgatatattgtacgggattaagcgaaagtattaagtgagccacctggggagtacgtcggcaacgatgaaactcaaaggaattgacggggcccgcacaagcggaggaacatgtggtttaattcgatgatacgcgaggaaccttacctgggtttaaatgggaatgtcgtatttgggaacagatattctcttcgagcgtttttcaaggtgctgcatggttgtcgtcagctcgtgcggtgaggggtcggtagtccata

SEQ ID NO: 25 - DNA, 982 bp, Artificial Sequence
  Synthetic Polynucleotide
ttttcttcggaactgaagatttggtgattgagtggcggacgggtgagtaacgcgtgggtaacctgccctgtacagggggataacagtcagaaatgactgctaataccgcataagaccacagcaccgcatggtgcaggggtaaaaactccggtggtacaggatggacccgcgtctgattagctggttggtgaggtaacggctcaccaaggcgacgatcagtagccggcttgagagagtgaacggccacattgggactgagacacggcccaaactcctacgggaggcagcagtggggaatattgcacaatgggggaaaccctgatgcagcgacgccgcgtgagtgaagaagtatctcggtatgtaaagctctatcagcagggaagaaaatgacggtacctgactaagaagccccggctaactacgtgccagcagccgcggtaatacgtagggggcaagcgttatccggaattactgggtgtaaagggtgcgtaggtggtatggcaagtcagaagtgaaaacccagggcttaactctgggactgcttttgaaactgtcagactggagtgcaggagaggtaagcggaattcctagtgtagcggtgaaatgcgtagatattaggaggaacatcagtggcgaaggcggcttactggactgaaactgacactgaggcacgaaagcgtggggagcaaacaggattagataccctggtagtccacgccgtaacgatgaatactaggtgtcggggccgtagaggcttcggtgccgcagccaacgcagtaagtattccacctggggagtacgttcgcaagaatgaaactcaaaggaattgacggggacccgcacaagcggtggagcatgtggtttattcgaagcaacgcgaagaaccttacctggtcttgacatccttctgaccggtccttaaccggactttccttcgggacagagtgacaaggtggtgcatgtgtcgtcagctcgtgtctga

SEQ ID NO: 26 - DNA, 387 bp, Artificial Sequence
  Synthetic Polynucleotide
agcaatactttgggtggcgaccggcgcacgggtgcgtaacgcgtatgtaacctacctataacaggggcataacactgagaaattggtactaattccccataatattcggagaggcatctctccgggttgaaaactccggtggttatagatggacatgcgttgtattagctagttggtgaggtaacggctcaccaaggcaacgatacatagggggactgagaggttaaccccccacactggtactgagacacggaccagactcctacgggaggcagcagtgaggaatattggtcaatggacgcaagtctgaaccagccaggccgcgtgcaggaagacggctctatgagttgtaaactgcttttgtacgagggtaaactcacctacgtg

SEQ ID NO: 27 - DNA, 843 bp, Artificial Sequence
  Synthetic Polynucleotide
attgtatcgcaaactcctagtaatcatcgtttactgcgtggactaccagggtatctaatcctgtttgatccccacgctttcgtgcttcagtgtcagttatggtttagtaagctgccttcgcaatcggagttctgcgtgatatctatgcatttcaccgctacaccacgcattccgcctacctcaaacacactcaagtaacccagtttcaacggcaattttatggttgagccacaaactttcaccgctgacttaaatcaccacctacgcaccctttaaacccaataaatccggataacgctcgcatcctccgtattaccgcggctgctggcacggagttagccgatgcttattcatagggtacatacaaaaaaggacacgtcctccactttattcccctataaaagaagtttacaaaccatagatccttcttccttcacgcgacttggctggttcagcctctcggccattgaccaatattcctcactgctgcctcccgtaggagtttggtccgtgtctcagtaccaatgtgggggaccttcctctcagaacccctatccatcgtcggtttggtgggccgttaccccgccaactgcctaatggaacgcatgcctatctatcagcgatgaatctttaacaaatattcccatgcgggacccctgttttatggggtattaatccgactttcgccgggctatccccctctgataggtaagttgcatacgcgttactcacccgtgcgccggtcgccatcaatctgtattgctacaaatcatgctgcccctcgacttgcatgtgttaagcctgtcgctagcgttcatcctgagccagattcaaactctataa

SEQ ID NO: 28 - DNA, 939 bp, Artificial Sequence
  Synthetic Polynucleotide
gaagcttcggcagatttggccggtttctagtggcggacgggtgagtaacgcgtgggtaacctgccttatacagggggataacaaccagaaatggttgctaataccgcataagcgcacaggaccgcatggtccagtgtgaaaaactccggtggtataagatggacccgcgttggattagctagttggcagggtaacggcctaccaaggcgacgatccatagccggcctgagagggtgaacggccacattgggactgagacacggcccagactcctacgggaggcagcagtggggaatattgcacaatgggggaaaccctgatgcagcgacgccgcgtgaaggaagaagtatctcggtatgtaaacttctatcagcagggaagatagtgacggtacctgactaagaagccccggctaactacgtgccagcagccgcggtaatacgtagggggcaagcgttatccggatttactgggtgtaaagggagcgtagacggactggcaagtctgatgtgaaaggcgggggctcaacccctggactgcattggaaactgttagtcttgagtgccggagaggtaagcggaattcctagtgtagcggtgaaatgcgtagatattaggaggaacaccagtggcgaaggcggcttactggacggtaactgacgttgaggctcgaaagcgtggggagcaaacaggattagataccctgggtagtccacgccgtaaacgatgaatactaggtgttgggggagcaaagctcttcggtgccgccgcaaacgcattaagtattccacctggggagtacgttcgcaagaatgaaactcaaaggatttgacggggacccgcacaagcgtggagcatgtgtttattcgaagcaaccggaagaacttaccaggcttgacatcctctgacgttcgtaacggaactttcttcggacaggaaa

SEQ ID NO: 29 - DNA, 956 bp, Artificial Sequence
  Synthetic Polynucleotide
tgctaaggccgatggcgaccggcgcacgggtgagtaacacgtatccaacctgccgtctactcttggacagccttctgaaaggaagattaatacaagatggcatcatgagtccgcatgttcacatgattaaaggtattccggtagacgatggggatgcgttccattagatagtaggcggggtaacggcccacctagtcttcgatggataggggttctgagaggaaggtcccccacattggaactgagacacggtccaaactcctacgggaggcagcagtgaggaatattggtcaatgggcgcaggcctgaaccagccaagtagcgtgaaggatgactgccctatgggttgtaaacttcttttataaaggaataaagtcgggtatgtatacccgtttgcatgtactttatgaataaggatcggctaactccgtgccagcagccgcggtaatacggaggatccgagcgttatccggatttattgggtttaaagggagcgtagatggatgtttaagtcagttgtgaaagtttgcggctcaaccgtaaaattgcagttgatactggatatcttgagtgcagttgaggcaggcggaattcgtggtgtagcggtgaaatgcttagatatcacgaagaactccgattgcgaaggcagcctgctaagctgcaactgacattgaggctcgaaagtgtgggtatcaaacaggattagataccctggtagtccacacggtaaacgatgaatactcgctgtttgcgatatacggcaagcggccaagcgaaagcgttaagtattccacctggggagtacgccggcaacggtgaactcaaaggaattgacggggcccgcacaagcggagaacatgtggtttaattcgatgatacgcgaggaccttacccggcttaaattgcagatgaattacgtgaagccgtaagccgcaagcatctgtgaagtgctgcat

SEQ ID NO: 30 - DNA, 980 bp, Artificial Sequence
  Synthetic Polynucleotide
taggttgatggcgaccggcgcacgggtgagtaacacgtatccaacctaccggttattccgggatagcctttcgaaagaaagattaataccggatagtataacgagaaggcatctttttgttattaaagaatttcgataaccgatggggatgcgttccattagtttgttggcggggtaacggcccaccaagacatcgatggataggggttctgagaggaaggtcccccacattggaactgagacacggtccaaactcctacgggaggcagcagtgaggaatattggtcaatggacgagagtctgaaccagccaagtagcgtgaaggatgactgccctatgggttgtaaacttcttttatatgggaataaagtgagccacgtgtggctttttgtatgtaccatacgaataaggatcggctaactccgtgccagcagccgcggtaatacggaggatccgagcgttatccggatttattgggtttaaagggagcgtaggcggactattaagtcagctgtgaaagtttgcggctcaaccgtaaaattgcagttgatactggtcgtcttgagtgcagtagaggtaggcggaattcgtggtgtagcggtgaaatgcttagatatcacgaagaactccgattgcgaaggcagcttactggactgtaactgacgctgatgctcgaaagtgtgggtatcaaacaggattagataccctggtagtccacacagtaaacgatgaatactcgctgtttgcgatatacagcaagcggccaagcgaaagcattaagtattccacctggggagtacgccggcaacggtgaaactcaaaggaattgacgggggcccgcacaagcgagaacatgtggtttaattcgatgatacgcgagaaccttaccgggcttaaattgcatctgaataatttggaaacagattagccgcaagcagatgtgaaggtgctgcatggtgtcgtcagctcgtgcgtgaggt

SEQ ID NO: 31 - DNA, 867 bp, Artificial Sequence
  Synthetic Polynucleotide
tgcttcaattgccggcgaccggcgcacgggtgcgtaacgcgtatgtaacctacctataacaggggcataacactgagaaattggtactaattccccataatattcggagaggcatctctccgggttgaaaactccggtggttatagatggacatgcgttgtattagctagttggtgaggtaacggctcaccaaggcaacgatacatagggggactgagaggttaaccccccacactggtactgagacacggaccagactcctacgggaggcagcagtgaggaatattggtcaatggacgcaagtctgaaccagccatgccgcgtgcaggaagacggctctatgagttgtaaactgcttttgtacgagggtaaactcacctacgtgtaggtgactgaaagtatcgtacgaataaggatcggctaactccgtgccagcagccgcggtaatacggaggattcaagcgttatccggatttattgggtttaaagggtgcgtaggcggtttgataagttagaggtgaaatcccggggcttaactccggaactgcctctaatactgttagactagagagtagttgcggtaggcggaatgtatggtgtagcggtgaaatgcttagagatcatacagaacaccgattgcgaaggcagcttaccaaactatatctgacgttgaggcacgaaagcgtggggagcaaaacaggattagataccctggtagtccacgcagtaaacgatgataactcgttgtcggcgatacacagtcggtgactaagcgaaagcgataagttatccacctggggagtacgttcgcaagaatgaacttaaaggaattgacggggcccgcacaagcggagaactgtggttatt

SEQ ID NO: 32 - DNA, 261 bp, Artificial Sequence
  Synthetic Polynucleotide
ttgctaagtttgatggcgaccggcgcacgggtgagtaacacgtatccaacctgccgatgactcggggatagcctttcgaaagaaagattaatacccgatggcatatttcttccgcatggtagaattattaaagaatttcggtcatcgatggggatgcgttccattaggttgttggcggggtaacggcccaccaagccttcgatggataggggttctgagaggaaggtcccccacattggaactgagccaggatcccaccat

SEQ ID NO: 33 - DNA, 832 bp, Artificial Sequence
  Synthetic Polynucleotide
gtgtatcgccgacaacgagttatcatcgtttactgcgtggactaccagggtatctaatcctgtttgctccccacgctttcgtgcctcaacgtcagatatagtttggtaagctgccttcgcaatcggtgttctgtatgatctctaagcatttcaccgctacaccatacattccgcctaccgcaactactctctagtctaacagtattagaggcagttccggagttaagccccgggatttcacctctaacttatcaaaccgcctacgcaccctttaaacccaataaatccggataacgcttgaatcctccgtattaccgcggctgctggcacggagttagccgatccttattcgtacgatactttcagtcacctacacgtaggtgagtttaccctcgtacaaaagcagtttacaactcatagagccgtcttcctgcacgcggcatggctggttcagacttgcgtccattgaccaatattcctcactgctgcctcccgtaggagtctggtccgtgtctcagtaccagtgtggggggttaacctctcagtccccctatgtatcgttgccttggtgagccgttacctcaccaactagctaatacaacgcatgtccatctataaccaccggagttttcaacccggagagatgcctctccgaatattatggggaattagtaccaatttctcagtgttatgcccctgttataggtaggttacatacgcgttacgcacccgtgcgccggtcgccaccaaagtattgctacctcgtgatgcccctcgacttgcatgtgttaggcctgccgctagcgttcatcctgagccagattcaaactct

SEQ ID NO: 34 - DNA, 1527 bp, Artificial Sequence
  Synthetic Polynucleotide
tcagagagtttgatcctggctcaggatgaacgctggcggcgtgcttaacacatgcaagtcgaacgggaaaccttttattgaagcttcggcagatttagattgtttctagtggcggacgggtgagtaacgcgtgggtaacctgccttatacagggggataacagtcagaaatgactgctaataccgcataagcgcacagagctgcatggctcggtgtgaaaaactccggtggtataagatggacccgcgttggattagctagttggtgaggtaacggcccaccaaggcgacgatccatagccggcctgagagggtgaacggccacattgggactgagacacggcccagactcctacgggaggcagcagtggggaatattgcacaatgggggaaaccctgatgcagcgacgccgcgtgaaggaagaagtatctcggtatgtaaacttctatcagcagggaagaaaatgacggtacctgactaagaagccccggctaactacgtgccagcagccgcggtaatacgtagggggcaagcgttatccggatttactgggtgtaaagggagcgtagacggatggacaagtctgatgtgaaaggctggggctcaaccccgggactgcattggaaactgcccgtcttgagtgccggagaggtaagcggaattcctagtgtagcggtgaaatgcgtagatattaggaggaacaccagtggcgaaggcggcttactggacggtaactgacgttgaggctcgaaagcgtggggagcaaacaggattagataccctggtagtccacgcggtaaacgatgaatgctaggtgtcggggagcaaagctcttcggtgccgccgcaaacgcattaagcattccacctggggagtacgttcgcaagaatgaaactcaaaggaattgacggggacccgcacaagcggtggagcatgtggtttaattcgaagcaacgcgaagaaccttaccaagtcttgacatccttctgaccggaacttaaccgttccttcccttcggggcagaagtgacaggtggtgcatggttgtcgtcagctcgtgtcgtgagatgttgggttaagtcccgcaacgagcgcaacccctatcctcagtagccagcatataaggtgggcactctggggagactgccagggataacctggaggaaggcggggatgacgtcaaatcatcatgccccttatgatttgggctacacacgtgctacaatggcgtaaacaaagggaagcgaacctgcgagggtgggcaaatcccaaaaataacgtcccagttcggactgtagtctgcaacccgactacacgaagctggaatcgctagtaatcgcggatcagaatgccgcggtgaatacgttcccgggtcttgtacacaccgcccgtcacaccatgggagtcagtaacgcccgaagtcagtgacctaaccgcaaggaaggagctgccgaaggcgggaccgatgactggggtgaagtcgtaacaaggtagccgtatcggaaggtgcggctggatcacctccttt

SEQ ID NO: 35 - DNA, 1055 bp, Artificial Sequence
  Synthetic Polynucleotide
  misc_feature (868)..(868): n is a, c, g, or t
  misc_feature (917)..(917): n is a, c, g, or t
  misc_feature (925)..(925): n is a, c, g, or t
  misc_feature (984)..(986): n is a, c, g, or t
  misc_feature (1002)..(1002): n is a, c, g, or t
  misc_feature (1015)..(1015): n is a, c, g, or t
  misc_feature (1020)..(1020): n is a, c, g, or t
  misc_feature (1049)..(1049): n is a, c, g, or t
gaggggcatgccatgatggagtagtaatatctatggtggcagaccggcgcacgggtgcgtaacgcgtatgcaacctacctttaacagggggataacactgagaaattggtactaataccccataatatcatagaaggcatcttttatggttgaaaattccgatggttagagatgggcatgcgttgtattagctagttggtggggtaacggctcaccaaggcgacgatacatagggggactgagaggttaaccccccacactggtactgagacacggaccagactcctacgggaggcagcagtgaggaatattggtcaatggacgcaagtctgaaccagccatgccgcgtgcaggatgacggctctatgagttgtaaactgcttttgtacgagggtaaacgcagatacgtgtatctgtctgaaagtatcgtacgaataaggatcggctaactccgtgccagcagccgcggtaatacggaggattcaagcgttatccggatttattgggtttaaagggtgcgtaggcggtttgataagttagaggtgaaatttcggggctcaaccctgaacgtgcctctaatactgttgagctagagagtagttgcggtaggcggaatgtatggtgtagcggtgaaatgcttagagatcatacagaacaccgattgcgaaggcagcttaccaaactatatctgacgttgaggcacgaaagcgtggggagcaaacaggattagataccctggtagtccacgcagtaaacgatgataactcgttgtcggcgatacacagtcggtgactaagcgaaagcgataagttatccacctggggagtacgttcgcaagaatgaaactcaaaggaattgacgggggccncgcacaagcggaggaacatgtgggtttaattcgatgatacgcgaggaanccttaccncgggcttgaaagttagcgacgattcttgaaagaggatttcccttcggggcgcgaaactnnngctgcatggttgtcgncagctcgtgccgngaggngtcgggttaagtcccataacgagcgcacnccctac

SEQ ID NO: 36 - DNA, 988 bp, Artificial Sequence
  Synthetic Polynucleotide
  misc_feature (5)..(5): n is a, c, g, or t
acacntgcagtcgaggggcagcataatggatagcaatatctatggtggcgaccggcgcacgggtgcgtaacgcgtatgcaacctacctttaacagggggataacactgagaaattggtactaataccccataatatcatagaaggcatcttttatggttgaaaattccgatggttagagatgggcatgcgttgtattagctagttggtggggtaacggctcaccaaggcgacgatacatagggggactgagaggttaaccccccacactggtactgagacacggaccagactcctacgggaggcagcagtgaggaatattggtcaatggacgcaagtctgaaccagccatgccgcgtgcaggatgacggctctatgagttgtaaactgcttttgtacgagggtaaacgcagatacgtgtatctgtctgaaagtatcgtacgaataaggatcggctaactccgtgccagcagccgcggtaatacggaggattcaagcgttatccggatttattgggtttaaagggtgcgtaggcggtttgataagttagaggtgaaatttcggggctcaaccctgaacgtgcctctaatactgttgagctagagagtagttgcggtaggcggaatgtatggtgtagcggtgaaatgcttagagatcatacagaacaccgattgcgaaggcagcttaccaaactatatctgacgttgaggcacgaaagcgtggggagcaaacaggattagataccctggtagtccacgcagtaaacgatgataactcgttgtcggcgatacacagtcggtgactaagcgaaagcgataagttatccacctggggagtacgttcgcaagaatgaaactcaaaggaattgacgggggcccgcacaagcggaggaacatgtggtttaattcgatgatacgcgaggaaccttacccgggcttgaaagttagcgacgattcttgaaagaggatttccctttcggggcgcgaaact

SEQ ID NO: 37 - DNA, 1029 bp, Artificial Sequence
  Synthetic Polynucleotide
  misc_feature (5)..(5): n is a, c, g, or t
  misc_feature (989)..(991): n is a, c, g, or t
acacntggaagtcgaggggcagcataatggatagcaatatctatggtggcgaccggcgcacgggtgcgtaacgcgtatgcaacctacctttaacagggggataacactgagaaattggtactaataccccataatatcatagaaggcatcttttatggttgaaaattccgatggttagagatgggcatgcgttgtattagctagttggtggggtaacggctcaccaaggcgacgatacatagggggactgagaggttaaccccccacactggtactgagacacggaccagactcctacgggaggcagcagtgaggaatattggtcaatggacgcaagtctgaaccagccatgccgcgtgcaggatgacggctctatgagttgtaaactgcttttgtacgagggtaaacgcagatacgtgtatctgtctgaaagtatcgtacgaataaggatcggctaactccgtgccagcagccgcggtaatacggaggattcaagcgttatccggatttattgggtttaaagggtgcgtaggcggtttgataagttagaggtgaaatttcggggctcaaccctgaacgtgcctctaatactgttgagctagagagtagttgcggtaggcggaatgtatggtgtagcggtgaaatgcttagagatcatacagaacaccgattgcgaaggcagcttaccaaactatatctgacgttgaggcacgaaagcgtggggagcaaacaggattagataccctggtagtccacgcagtaaacgatgataactcgttgtcggcgatacacagtcggtgactaagcgaaagcgataagttatccacctggggagtacgttcgcaagaatgaaactcaaaggaattgacgggggcccgcacaagcggaggaacatgtggtttaattcgatgatacgcgaggaaccttacccgggcttgaaagttagcgacgattcttgaaagaggatttcccttcggggcgcgaaactnnngctgcatggtgtcgtcagctcgtgccgtgaggtgtcgg